European Patent Application EP 4 465 043 A1, published November 20, 2024. Title: A method for detecting an antibody to Helicobacter suis using solubilized fraction of bacteria. Applicant: Kitasato Institute. The sequence listing filed with the application follows.

SEQUENCE LISTING (11 sequences)

SEQ ID NO: 1 - protein, 14 aa, synthetic construct
  REGION 1..14: note = Synthetic
EKKAVQQMENSNPD

SEQ ID NO: 2 - protein, 14 aa, synthetic construct
  REGION 1..14: note = Synthetic
EKKAVEQMENSNPD

SEQ ID NO: 3 - protein, 14 aa, synthetic construct
  REGION 1..14: note = Synthetic
EKDAVTSLKNSNSG

SEQ ID NO: 4 - protein, 14 aa, synthetic construct
  REGION 1..14: note = Synthetic
EKDAVTSLENSNSG

SEQ ID NO: 5 - protein, 14 aa, synthetic construct
  REGION 1..14: note = Synthetic
NQGTLEFLSNDVST

SEQ ID NO: 6 - protein, 14 aa, synthetic construct
  REGION 1..14: note = Synthetic
TNGQEVSASIDYNK

SEQ ID NO: 7 - protein, 14 aa, synthetic construct
  REGION 1..14: note = Synthetic
AKLSNFASNDALPD

SEQ ID NO: 8 - protein, 14 aa, synthetic construct
  REGION 1..14: note = Synthetic
PTTSSGASPDSSNP

SEQ ID NO: 9 - protein, 14 aa, synthetic construct
  REGION 1..14: note = Synthetic
NVDNILNMPSTTSG

SEQ ID NO: 10 - protein, 14 aa, synthetic construct
  REGION 1..14: note = Synthetic
TLTLEGTETFAQNS

SEQ ID NO: 11 - protein, 14 aa, synthetic construct
  REGION 1..14: note = Synthetic
ADIQSSQTTFANSV